European Patent Application EP 4 474 393 A1, published December 11, 2024. Title: Broadly neutralizing antibodies targeting the CD4 binding site on HIV Env. Applicant: Universität zu Köln. The sequence listing filed with the application follows.

SEQUENCE LISTING (40 sequences)

SEQ ID NO: 1 - protein, 19 aa, synthetic construct
DSFTVYRPRLSAYFIGEFN

SEQ ID NO: 2 - protein, 8 aa, synthetic construct
VNIFRGAV

SEQ ID NO: 3 - protein, 15 aa, synthetic construct
AWDKNVDDNPWRLDS

SEQ ID NO: 4 - protein, 6 aa, synthetic construct
QDVGWA

SEQ ID NO: 5 - skipped

SEQ ID NO: 6 - protein, 5 aa, synthetic construct
QVFDS

SEQ ID NO: 7 - protein, 8 aa, synthetic construct
GYSFRDYR

SEQ ID NO: 8 - protein, 8 aa, synthetic construct
MQPRYGAV

SEQ ID NO: 9 - protein, 20 aa, synthetic construct
VTHKLYDGEDASDLTWRLDP

SEQ ID NO: 10 - protein, 6 aa, synthetic construct
QDITNA

SEQ ID NO: 11 - skipped

SEQ ID NO: 12 - protein, 5 aa, synthetic construct
QHYEF

SEQ ID NO: 13 - protein, 8 aa, synthetic construct
AYFIGEFN

SEQ ID NO: 14 - protein, 8 aa, synthetic construct
VNIFRGAV

SEQ ID NO: 15 - protein, 15 aa, synthetic construct
AWDKNVDDNPWRLDS

SEQ ID NO: 16 - protein, 6 aa, synthetic construct
QDVGWA

SEQ ID NO: 17 - skipped

SEQ ID NO: 18 - protein, 5 aa, synthetic construct
QVFES

SEQ ID NO: 19 - protein, 8 aa, synthetic construct
GYTFRDYR

SEQ ID NO: 20 - protein, 8 aa, synthetic construct
LHPAYGAV

SEQ ID NO: 21 - protein, 20 aa, synthetic construct
VTHKLYDGEDASDLTWRLDP

SEQ ID NO: 22 - protein, 6 aa, synthetic construct
QDITNA

SEQ ID NO: 23 - skipped

SEQ ID NO: 24 - protein, 5 aa, synthetic construct
QHYEF

SEQ ID NO: 25 - protein, 8 aa, synthetic construct
GYSFRDYR

SEQ ID NO: 26 - protein, 8 aa, synthetic construct
IQPRYGAV

SEQ ID NO: 27 - protein, 20 aa, synthetic construct
VTHKLYDGEDASDLAWRLDP

SEQ ID NO: 28 - protein, 6 aa, synthetic construct
QDITNA

SEQ ID NO: 29 - skipped

SEQ ID NO: 30 - protein, 5 aa, synthetic construct
QHYEF

SEQ ID NO: 31 - protein, 133 aa, synthetic construct
SVRLDQSGTAVKKPGASVRVSCRAPDSFTVYRPRLSAYFIGEFNIHWLRQAPGQGLEWLGFVNIFRGAVKYSSRFQGRITITRDTSSETSYLDLGALKADDTATYYCAWDKNVDDNPWRLDSWGQGTLVIVSS

SEQ ID NO: 32 - protein, 103 aa, synthetic construct
YIQVTQSPSSLSASIGDTITVACEVSQDVGWAVNWYHQRPGRPPYNLIYTAHNLAPGVASRFRGSRVGTYFTLTINNLLPEDVGTYYCQVFDSFAPGGTRVDL

SEQ ID NO: 33 - protein, 137 aa, synthetic construct
HVQLWQSGAEVKKPGASVKISCSAWGFGTTSGYSFRDYRVHWVRHIAGQGFQWMGHMQPRYGAVNYARQFQGRITMTREVSFDASGGTAYMELRSLRSDDTAVYYCVTHKLYDGEDASDLTWRLDPWGQGTRVIVSS

SEQ ID NO: 34 - protein, 104 aa, synthetic construct
GVHLTQSPASLSASVGDRVTFTCQASQDITNAINWYQLRPGKTPKLMIHDGSTLRRGVPSRFAGSGFGTKFTFTIDNLQPEDLATYFCQHYEFFPPVGTQVELN

SEQ ID NO: 35 - protein, 133 aa, synthetic construct
SVRLDQSGTAVKKPGASVRVSCRAPDSFTVYRPRLSAYFIGEFNIHWLRQAPGQGLEWLGFVNIFRGAVKYSSAFRGRITITRDTSLETSYLDLGALKPDDTATYFCAWDKNVDDNPWRLDSWGQGTLVVVSS

SEQ ID NO: 36 - protein, 104 aa, synthetic construct
YIQVTQSPSSLSASVGDTITVACQVSQDVGWAVNWYHQRPGRPPYNLIYTTSNLAPGVASRFRGTRVATYFTLTINNLLPEDVGTYYCQVFESFAPGGTRVDLR

SEQ ID NO: 37 - protein, 137 aa, synthetic construct
HVQLWQSGAEVKKPGASVKISCSAWGFGTRSGYTFRDYRIHWVRQVPRQGFEWMGHLHPAYGAVNYARQFQGRIIMTREVSFDGSGGTVYMELRSLRSDDTATYYCVTHKLYDGEDASDLTWRLDPWGQGTRVTVSS

SEQ ID NO: 38 - protein, 104 aa, synthetic construct
GVSLTQSPASLCASVGDRVTFTCQASQDITNAINWYQLRPGKTPKLMIHDGSTLRRGVPSRFAGSGFGTRFTFTIDNLQPEDLATYFCQHYEFFPPAGTQVDFN

SEQ ID NO: 39 - protein, 137 aa, synthetic construct
HVQLWQSGAEVKKPGASVKISCAAWGFGTTSGYSFRDYRIHWVRQVPGQGFQWMGHIQPRYGAVNYAHQFQGRITMTREVSFDASGGTAYMELRSLRSDDTATYYCVTHKLYDGEDASDLAWRLDPWGQGTRVTVSS

SEQ ID NO: 40 - protein, 104 aa, synthetic construct
GVHLTQSPASLSASVGDRVTFTCQASQDITNAINWYQLRPGKTPKLMIHDGSTLRRGVPSRFAGGGFGTKFTFTIDNLQPEDLATYFCQHYEFFPPAGTQVELN